European Patent Specification EP 3 390 429 B1, published June 18, 2025. Title: MODIFIED CAPSID PROTEINS FOR ENHANCED DELIVERY OF PARVOVIRUS VECTORS. Applicant: The University of North Carolina at Chapel Hill Samulski, Richard Jude Warishalk, Jayme. The sequence listing filed with the application follows.

SEQUENCE LISTING (48 sequences)

SEQ ID NO: 1 - protein, 13 aa, adeno-associated virus 1
SSASTGASNDNHY

SEQ ID NO: 2 - protein, 7 aa, adeno-associated virus 2
SSQSGAS

SEQ ID NO: 3 - protein, 12 aa, adeno-associated virus 3B
SSQSGASNDNHY

SEQ ID NO: 4 - protein, 8 aa, adeno-associated virus 4
ESLQSNTY

SEQ ID NO: 5 - protein, 7 aa, adeno-associated virus 5
SGSVDGS

SEQ ID NO: 6 - protein, 13 aa, adeno-associated virus 6
SSASTGASNDNHY

SEQ ID NO: 7 - protein, 8 aa, adeno-associated virus 8
NGTSGGAT

SEQ ID NO: 8 - protein, 9 aa, adeno-associated virus 9
SNSTSGGSS

SEQ ID NO: 9 - DNA, 24 bp, Artificial
  Quantitative PCR primer sequence
aaaagcactctgattgacaaatac

SEQ ID NO: 10 - DNA, 22 bp, Artificial
  Quantitative PCR primer sequence
ccttcgcttcaaaaaatggaac

SEQ ID NO: 11 - DNA, 19 bp, Artificial
  Quantitative PCR primer sequence
aagtcaaggacaccgagga

SEQ ID NO: 12 - DNA, 20 bp, Artificial
  Quantitative PCR primer sequence
cccagctggacagtctctta

SEQ ID NO: 13 - DNA, 34 bp, Artificial
  Site-directed mutagenesis primer sequence
gcaatctccagtgcttcagacggggccagcaacg

SEQ ID NO: 14 - DNA, 35 bp, Artificial
  Site-directed mutagenesis primer sequence
  misc_feature (13)..(13): n is a, c, g, or t
gcaatctccagtngcttcagagggggccagcaacg

SEQ ID NO: 15 - DNA, 36 bp, Artificial
  Site-directed mutagenesis primer sequence
gcaatctccagtgcttcattcggggccagcaacgac

SEQ ID NO: 16 - DNA, 26 bp, Artificial
  Site-directed mutagenesis primer sequence
caagcaaatcagtgcttcaacggggg

SEQ ID NO: 17 - DNA, 23 bp, Artificial
  Site-directed mutagenesis primer sequence
gcaaatctccgcttcaacggggg

SEQ ID NO: 18 - DNA, 24 bp, Artificial
  Site-directed mutagenesis primer sequence
gcaaatctccagttcaacgggggc

SEQ ID NO: 19 - DNA, 30 bp, Artificial
  Site-directed mutagenesis primer sequence
caaatctccagtgctacgggggccagaaac

SEQ ID NO: 20 - DNA, 26 bp, Artificial
  Site-directed mutagenesis primer sequence
ctccagtgcttcaggggccagcaacg

SEQ ID NO: 21 - DNA, 23 bp, Artificial
  Site-directed mutagenesis primer sequence
ccagtgcttcaacggccgcaagc

SEQ ID NO: 22 - DNA, 25 bp, Artificial
  Site-directed mutagenesis primer sequence
gcttcaacggggagcaacgacaacc

SEQ ID NO: 23 - DNA, 20 bp, Artificial
  Site-directed mutagenesis primer sequence
cgggggccaacgacaaccac

SEQ ID NO: 24 - DNA, 23 bp, Artificial
  Site-directed mutagenesis primer sequence
cgggggccagcgacaaccacttc

SEQ ID NO: 25 - DNA, 23 bp, Artificial
  Quantitative PCR primer sequence
ggacccaaggactacctcaaggg

SEQ ID NO: 26 - DNA, 22 bp, Artificial
  Quantitative PCR primer sequence
agggcacctccatctcggaaac

SEQ ID NO: 27 - DNA, 26 bp, Artificial
  Quantitative PCR primer sequence
ctccagtgcttcaggggccagcaacg

SEQ ID NO: 28 - DNA, 36 bp, Artificial
  Quantitative PCR primer sequence
catcgaccagtacctgtatttcctgaacagaactca

SEQ ID NO: 29 - DNA, 28 bp, Artificial
  Quantitative PCR primer sequence
caaacaaatttccagctcaggagcctcg

SEQ ID NO: 30 - DNA, 28 bp, Artificial
  Quantitative PCR primer sequence
caaatttccagccaaggagcctcgaacg

SEQ ID NO: 31 - DNA, 27 bp, Artificial
  Quantitative PCR primer sequence
caagcaaatctccagctcaggagcttc

SEQ ID NO: 32 - DNA, 29 bp, Artificial
  Quantitative PCR primer sequence
ctccagccaatcagacggagcttcaaacg

SEQ ID NO: 33 - DNA, 30 bp, Artificial
  Quantitative PCR primer sequence
cagctcccacgactgcaactgtcaatgatc

SEQ ID NO: 34 - DNA, 24 bp, Artificial
  Quantitative PCR primer sequence
gagcctgcagtccacctacaacgg

SEQ ID NO: 35 - DNA, 23 bp, Artificial
  Quantitative PCR primer sequence
ccgtcgacggaaacgccaacgcc

SEQ ID NO: 36 - DNA, 23 bp, Artificial
  Quantitative PCR primer sequence
gcaaatctccgcttcaacggggg

SEQ ID NO: 37 - DNA, 27 bp, Artificial
  Quantitative PCR primer sequence
caaatctccagtgaagcaggtagtacc

SEQ ID NO: 38 - DNA, 21 bp, Artificial
  Quantitative PCR primer sequence
ctccaacgggtcgggaggagc

SEQ ID NO: 39 - DNA, 33 bp, Artificial
  Quantitative PCR primer sequence
caaatctccaacggggactcgggaggagccacc

SEQ ID NO: 40 - DNA, 27 bp, Artificial
  Quantitative PCR primer sequence
tctccaacgggacaggaggagccaacc

SEQ ID NO: 41 - DNA, 27 bp, Artificial
  Quantitative PCR primer sequence
caagcaaatctccagcacatctggagg

SEQ ID NO: 42 - DNA, 29 bp, Artificial
  Quantitative PCR primer sequence
ctccaacagcacaggaggatcttcaaatg

SEQ ID NO: 43 - DNA, 41 bp, Artificial
  Quantitative PCR primer sequence
caagcaaatctccaacagcgactctggaggatcttcaaatg

SEQ ID NO: 44 - DNA, 37 bp, Artificial
  Site-directed mutagenesis primer sequence
gcaaatctccaacgccacaggaggatcttcaaatgac

SEQ ID NO: 45 - DNA, 23 bp, Artificial
  Quantitative PCR primer sequence
ggacccaaggactacctcaaggg

SEQ ID NO: 46 - DNA, 22 bp, Artificial
  Quantitative PCR primer sequence
agggcacctccatctcggaaac

SEQ ID NO: 47 - protein, 8 aa, Artificial
  Mutated VR1 capsid amino acid sequence
  misc_feature (3)..(3): Xaa can be any naturally occurring amino acid
SSXSDGAS

SEQ ID NO: 48 - protein, 8 aa, Artificial
  Mutated VR1 capsid amino acid sequence
  misc_feature (3)..(3): Xaa can be any naturally occurring amino acid
SSXSDGAS